European Patent Application EP 4 659 762 A1, published December 10, 2025. Title: Pharmaceutical composition for the treatment of liver fibrosis. Applicant: 学校法人大阪医科薬科大学. The sequence listing filed with the application follows.

SEQUENCE LISTING (23 sequences)

SEQ ID NO: 1 - DNA, 18 bp, synthetic construct
  source 1..18: mol_type = other DNA
gaagcccgagaacatcat

SEQ ID NO: 2 - DNA, 18 bp, synthetic construct
  source 1..18: mol_type = other DNA
cagctagcagcaagcaca

SEQ ID NO: 3 - DNA, 18 bp, synthetic construct
  source 1..18: mol_type = other DNA
gatgatctgcatgtcttc

SEQ ID NO: 4 - DNA, 17 bp, synthetic construct
  source 1..17: mol_type = other DNA
tgtggtgatgatctgca

SEQ ID NO: 5 - DNA, 18 bp, synthetic construct
  source 1..18: mol_type = other DNA
gggctgtggtgatgatct

SEQ ID NO: 6 - DNA, 17 bp, synthetic construct
  source 1..17: mol_type = other DNA
aagcacaccagggctgt

SEQ ID NO: 7 - DNA, 20 bp, synthetic construct
  source 1..20: mol_type = other DNA
catctggagaagggtacctg

SEQ ID NO: 8 - DNA, 20 bp, synthetic construct
  source 1..20: mol_type = other DNA
cattggagcagatggagctg

SEQ ID NO: 9 - DNA, 20 bp, synthetic construct
  source 1..20: mol_type = other DNA
aagccatgtggtttccagag

SEQ ID NO: 10 - DNA, 20 bp, synthetic construct
  source 1..20: mol_type = other DNA
aaggaatggtgtagggctgg

SEQ ID NO: 11 - DNA, 20 bp, synthetic construct
  source 1..20: mol_type = other DNA
cagagggttgggggttgatg

SEQ ID NO: 12 - DNA, 18 bp, synthetic construct
  source 1..18: mol_type = other DNA
gccatgtggtttccagag

SEQ ID NO: 13 - DNA, 18 bp, synthetic construct
  source 1..18: mol_type = other DNA
gagaagggtacctgcatg

SEQ ID NO: 14 - DNA, 18 bp, synthetic construct
  source 1..18: mol_type = other DNA
caacatctggagaagggt

SEQ ID NO: 15 - DNA, 18 bp, synthetic construct
  source 1..18: mol_type = other DNA
gtcttctggtctggcttg

SEQ ID NO: 16 - DNA, 18 bp, synthetic construct
  source 1..18: mol_type = other DNA
atgtcttctggtctggct

SEQ ID NO: 17 - DNA, 18 bp, synthetic construct
  source 1..18: mol_type = other DNA
catgtcttctggtctggc

SEQ ID NO: 18 - DNA, 18 bp, synthetic construct
  source 1..18: mol_type = other DNA
tgtggtgatgatctgcat

SEQ ID NO: 19 - DNA, 18 bp, synthetic construct
  source 1..18: mol_type = other DNA
ctgtggtgatgatctgca

SEQ ID NO: 20 - DNA, 18 bp, synthetic construct
  source 1..18: mol_type = other DNA
agggctgtggtgatgatc

SEQ ID NO: 21 - DNA, 17 bp, synthetic construct
  source 1..17: mol_type = other DNA
gggctgtggtgatgatc

SEQ ID NO: 22 - DNA, 17 bp, synthetic construct
  source 1..17: mol_type = other DNA
agggctgtggtgatgat

SEQ ID NO: 23 - DNA, 18 bp, synthetic construct
  source 1..18: mol_type = other DNA
cagggctgtggtgatgat